European Patent Application EP 4 198 056 A1, published June 21, 2023. Title: ANTIBODY BINDING TO HUMAN CD38, PREPARATION METHOD THEREOF, AND USE THEREOF. Applicant: Sunshine Guojian Pharmaceutical (Shanghai) Co., Ltd. The sequence listing filed with the application follows.

SEQUENCE LISTING (22 sequences)

SEQ ID NO: 1 - protein, 5 aa, Mus musculus
TYWMQ

SEQ ID NO: 2 - protein, 17 aa, mus musculus
AIYPGDGDITYNQKFKG

SEQ ID NO: 3 - protein, 11 aa, mus musculus
EGYYYGGALDY

SEQ ID NO: 4 - protein, 12 aa, mus musculus
TASSSVSSSYLH

SEQ ID NO: 5 - protein, 7 aa, mus musculus
GTSNLAS

SEQ ID NO: 6 - protein, 9 aa, mus musculus
HRYHRSPWT

SEQ ID NO: 7 - protein, 120 aa, mus musculus
QVQLQQSGAELARPGASVKLSCKASGYTFNTYWMQWVKQRPGQGLEWIGAIYPGDGDITYNQKFKGKATLTADKSSNTAYMHLSSLASEDSAVYYCAREGYYYGGALDYWGQGTSVTVSS

SEQ ID NO: 8 - protein, 108 aa, mus musculus
QIFLTQSPAIMSASLGERVTMTCTASSSVSSSYLHWYQQKPGSPPKLWMYGTSNLASGVPPRFSGSGSGTSYSLTISSMEAEDAATYYCHRYHRSPWTFGGGTKLEIK

SEQ ID NO: 9 - protein, 120 aa, Artificial Sequence
  CD38 humanized antibody heavy chain variable region 50G12-Hu-VH
QVQLVQSGAEVKKPGASVKVSCKASGYTFNTYWMQWVRQAPGQGLEWMGAIYPGDGDITYNQKFKGRVTLTADKSTSTVYMELSSLRSEDTAVYYCAREGYYYGGALDYWGQGTLVTVSS

SEQ ID NO: 10 - protein, 108 aa, Artificial Sequence
  CD38 humanized antibody light chain variable region 50G12-Hu-VL
DIQMTQSPSSLSASVGDRVTITCTASSSVSSSYLHWYQQKPGKAPKLWMYGTSNLASGVPSRFSGSGSGTDYTLTISSLQPEDFATYYCHRYHRSPWTFGQGTKVEIK

SEQ ID NO: 11 - protein, 450 aa, Artificial Sequence
  CD38 humanized antibody heavy chain 50G12-Hu-HC
QVQLVQSGAEVKKPGASVKVSCKASGYTFNTYWMQWVRQAPGQGLEWMGAIYPGDGDITYNQKFKGRVTLTADKSTSTVYMELSSLRSEDTAVYYCAREGYYYGGALDYWGQGTLVTVSSASTKGPSVFPLAPSSKSTSGGTAALGCLVKDYFPEPVTVSWNSGALTSGVHTFPAVLQSSGLYSLSSVVTVPSSSLGTQTYICNVNHKPSNTKVDKKVEPKSCDKTHTCPPCPAPELLGGPSVFLFPPKPKDTLMISRTPEVTCVVVDVSHEDPEVKFNWYVDGVEVHNAKTKPREEQYNSTYRVVSVLTVLHQDWLNGKEYKCKVSNKALPAPIEKTISKAKGQPREPQVYTLPPSREEMTKNQVSLTCLVKGFYPSDIAVEWESNGQPENNYKTTPPVLDSDGSFFLYSKLTVDKSRWQQGNVFSCSVMHEALHNHYTQKSLSLSPGK

SEQ ID NO: 12 - protein, 215 aa, Artificial Sequence
  CD38 humanized antibody light chain 50G12-Hu-LC
DIQMTQSPSSLSASVGDRVTITCTASSSVSSSYLHWYQQKPGKAPKLWMYGTSNLASGVPSRFSGSGSGTDYTLTISSLQPEDFATYYCHRYHRSPWTFGQGTKVEIKRTVAAPSVFIFPPSDEQLKSGTASVVCLLNNFYPREAKVQWKVDNALQSGNSQESVTEQDSKDSTYSLSSTLTLSKADYEKHKVYACEVTHQGLSSPVTKSFNRGEC

SEQ ID NO: 13 - DNA, 360 bp, mus musculus
caggttcagctccagcagtctggggctgagctggcaagacctggggcctcagtgaagttgtcctgcaaggcttctggctacacctttaatacctattggatgcagtgggtaaaacagaggcctggacagggtctggaatggattggggctatttatcctggagatggtgatattacatataatcagaagtttaagggcaaggccacattgactgcagataaatcttccaacacagcctacatgcacctcagcagcttggcatctgaggactcagcggtctattactgtgcaagagagggatattattacggcggggctttggactactggggtcaaggaacctcagtcaccgtctcctca

SEQ ID NO: 14 - DNA, 324 bp, mus musculus
caaatttttctcacccagtctccagcaatcatgtctgcatctctaggggaacgggtcaccatgacctgcactgccagctcaagtgtgagttcaagctacttgcactggtaccagcagaagccaggatccccccccaaactctggatgtatggcacatccaacctggcttctggagtcccacctcgcttcagtggcagtgggtctgggacctcttactctctcacaatcagcagcatggaggctgaagatgctgccacttattactgccaccggtatcatcgttccccgtggacgttcggtggaggcaccaagctggaaatcaaa

SEQ ID NO: 15 - DNA, 360 bp, Artificial Sequence
  50G12-Hu-VH heavy chain variable region nucleotide sequence
caggtgcagctcgtgcagtccggcgctgaggtgaagaagcccggcgcctccgtgaaggtgtcctgcaaggcctccggctacaccttcaacacctattggatgcaatgggtgaggcaggcccccggccagggcctggagtggatgggcgccatctaccccggcgatggcgacatcacctacaaccagaagtttaagggcagggtgaccctgacagctgataaatctacatctactgtgtacatggagttatcttctctgagatctgaggatacagctgtgtactattgtgctagagagggatactattatggcggagccctggattattggggacagggaacactggtgacagtgtcttct

SEQ ID NO: 16 - DNA, 324 bp, Artificial Sequence
  50G12-Hu-LC light chain variable region nucleotide sequence
gatatccagatgacccagtctccttcttccctgtccgcttctgtgggagatagagtgacaattacatgtaccgcttcttcttctgtgtcttcttcttacctgcattggtatcagcagaagcctggcaaggctcctaaactgtggatgtatggaacatctaatctggcttctggcgtgccttctagattttctggctctggatctggcaccgattacacactgaccatctctagcctgcagcctgaggattttgccacatactactgtcacagatatcacagatctccttggacctttggccagggcaccaaggtggagatcaag

SEQ ID NO: 17 - DNA, 1350 bp, Artificial Sequence
  50G12-Hu-HC heavy chain nucleotide sequence
caggtgcagctcgtgcagtccggcgctgaggtgaagaagcccggcgcctccgtgaaggtgtcctgcaaggcctccggctacaccttcaacacctattggatgcaatgggtgaggcaggcccccggccagggcctggagtggatgggcgccatctaccccggcgatggcgacatcacctacaaccagaagtttaagggcagggtgaccctgacagctgataaatctacatctactgtgtacatggagttatcttctctgagatctgaggatacagctgtgtactattgtgctagagagggatactattatggcggagccctggattattggggacagggaacactggtgacagtgtcttctgcgagcaccaagggaccttccgtgtttcccctcgcccccagctccaaaagcaccagcggcggaacagctgctctcggctgtctcgtcaaggattacttccccgagcccgtgaccgtgagctggaacagcggagccctgacaagcggcgtccacaccttccctgctgtcctacagtcctccggactgtacagcctgagcagcgtggtgacagtccctagcagctccctgggcacccagacatatatttgcaacgtgaatcacaagcccagcaacaccaaggtcgataagaaggtggagcctaagtcctgcgacaagacccacacatgtcccccctgtcccgctcctgaactgctgggaggcccttccgtgttcctgttcccccctaagcccaaggacaccctgatgatttccaggacacccgaggtgacctgtgtggtggtggacgtcagccacgaggaccccgaggtgaaattcaactggtacgtcgatggcgtggaggtgcacaacgctaagaccaagcccagggaggagcagtacaattccacctacagggtggtgtccgtgctgaccgtcctccatcaggactggctgaacggcaaagagtataagtgcaaggtgagcaacaaggccctccctgctcccatcgagaagaccatcagcaaagccaagggccagcccagggaacctcaagtctataccctgcctcccagcagggaggagatgaccaagaaccaagtgagcctcacatgcctcgtcaagggcttctatccttccgatattgccgtcgagtgggagtccaacggacagcccgagaacaactacaagacaacaccccccgtgctcgattccgatggcagcttcttcctgtactccaagctgaccgtggacaagtccagatggcaacaaggcaacgtcttcagttgcagcgtcatgcatgaggccctccacaaccactacacccagaagagcctctccctgagccctggaaag

SEQ ID NO: 18 - DNA, 645 bp, Artificial Sequence
  50G12-Hu-HC light chain nucleotide sequence
gatatccagatgacccagtctccttcttccctgtccgcttctgtgggagatagagtgacaattacatgtaccgcttcttcttctgtgtcttcttcttacctgcattggtatcagcagaagcctggcaaggctcctaaactgtggatgtatggaacatctaatctggcttctggcgtgccttctagattttctggctctggatctggcaccgattacacactgaccatctctagcctgcagcctgaggattttgccacatactactgtcacagatatcacagatctccttggacctttggccagggcaccaaggtggagatcaagagaaccgtcgccgctcccagcgtcttcatcttcccccccagcgatgagcagctgaagagcggaaccgccagcgtggtgtgcctgctgaacaacttctaccccagggaggccaaggtgcaatggaaggtggacaacgccctacagagcggcaactcccaggagagcgtgaccgagcaggacagcaaggatagcacctacagcctgagcagcaccctcaccctgagcaaggccgactacgagaagcacaaggtgtacgcctgcgaggtgacccatcagggcctgagcagccctgtgaccaagagcttcaacaggggcgagtgc

SEQ ID NO: 19 - protein, 122 aa, Artificial Sequence [sequence omitted]

SEQ ID NO: 20 - protein, 107 aa, Artificial Sequence [sequence omitted]

SEQ ID NO: 21 - protein, 120 aa, Artificial Sequence [sequence omitted]

SEQ ID NO: 22 - protein, 107 aa, Artificial Sequence [sequence omitted]